European Patent Application EP 4 748 843 A2, published May 27, 2026. Title: ANTIBODY-DRUG CONJUGATE, AND PREPARATION METHOD THEREFOR AND USE THEREOF. Applicant: Medilink Therapeutics (SuZhou) Co., Ltd. The sequence listing filed with the application follows.

SEQUENCE LISTING (87 sequences)

SEQ ID NO: 1 - protein, 119 aa, synthetic construct
QVQLQQSGPVLVKPGASVKMSCKASGYTFTDYYMNWVKQSHGKSLEWIGVINPYNGGTNYSQKFKGKATLTVDKSSSTAYMELNSLTSEDSAVYYCARDSNYVGLLDYWGQGTSVTVSS

SEQ ID NO: 2 - protein, 113 aa, synthetic construct
QVQLVESGAEVKKPGSSVKVSCKASGYAFSSHWVNWVRQAPGQGLEWMGQIYPGNGDTNYAQKFQGRVTLTADKSTSTAYMELSSLTSEDTAVYFCARWFAYWGQGTLVTVSS

SEQ ID NO: 3 - protein, 113 aa, synthetic construct
DIVMTQSPSSLAMSVGQRVTINCKSSQSLLDGGNQKNYLAWYQQKVGQPPKLLVYFASIRESGVPDRFIGSGSGTDFTLTISSVQTEDLADYFCQQHYNTPWTFGGGTKLEIK

SEQ ID NO: 4 - protein, 113 aa, synthetic construct
DIQMTQSPSSLSASVGDRVTITCKSSQSLLDGGNQKNYLAWYQQKPGKPPKLLVYFASIRESGVPSRFSGSGSGTDFTLTISSLQPEDFATYYCQQHYNTPWTFGQGTKVEIK

SEQ ID NO: 5 - protein, 119 aa, synthetic construct
EVQLQQSGPVLVKPGASVKMSCKASGYTFTDYYMNWVKQSHGKSLEWIGVINPYNGGTNYSQKFKGKATLTVDKSSSTAYMELNSLTSEDSAVYYCARDSNYVGLLDYWGQGTSVTVSS

SEQ ID NO: 6 - protein, 119 aa, synthetic construct
EVQLVQSGAEVKKPGASVKVSCKASGYTFTDYYMNWVRQAPGQRLEWMGVINPYNGGTNYSQKFQGRVTLTVDKSASTAYMELSSLRSEDTAVYYCARDSNYVGLLDYWGQGTLVTVSS

SEQ ID NO: 7 - protein, 119 aa, synthetic construct
EVQLVQSGAEVKKPGASVKVSCKASGYTFTDYYMNWVRQAPGQRLEWMGVINPYNGGTNYAQKFQGRVTLTVDKSASTAYMELSSLRSEDTAVYYCARDSNYVGLLDYWGQGTLVTVSS

SEQ ID NO: 8 - protein, 107 aa, synthetic construct
DIVLTQSPATLSVTPGDSVSLSCRASQSISNNLHWYQQKSHESPRLLIKYASQSISGIPSRFSGSGSGPDFTLSIDSVETEDFGVYFCQQSNSWPYTFGGGTKLEIK

SEQ ID NO: 9 - protein, 107 aa, synthetic construct
DIVLTQSPATLSLSPGERATLSCRASQSISNNLHWYQQKPGQAPRLLIKYASQSISGIPARFSGSGSGPDFTLTISSLEPEDFAVYFCQQSNSWPYTFGQGTKVEIK

SEQ ID NO: 10 - protein, 125 aa, synthetic construct
EVKLEESGGGLVQPGGSMKLSCAASGFTFSDAWMDWVRQSPEKGLEWIAEIRNKANNHATYYTESVKGRFTISRDDSKSSVYLQMISLRPEDTGIYYCTRNNYGSTWTYYAMDYWGQGTSVTVSS

SEQ ID NO: 11 - protein, 125 aa, synthetic construct
EVQLVESGGGLVQPGGSLRLSCAASGFTFSDAWMDWVRQAPGKGLEWVAEIRNKANNHATYYVDSVKGRFTISRDDAKNSVYLQMNSLRAEDTAVYYCTRNNYGSTWTYYAMDYWGQGTLVTVSS

SEQ ID NO: 12 - protein, 107 aa, synthetic construct
DIQMTQTSSSLSASLGDRVTINCRASQDISNYLNWYQQKPDGTVKLLIYYTSRLHSGVPSRFSGSGSGTDYSLTISNLEHEDIATYFCQQGYTLPLTFGAGTNLELK

SEQ ID NO: 13 - protein, 107 aa, synthetic construct
DIQMTQSPSSLSASVGDRVTITCRASQDISNYLNWYQQKPGKAVKLLIYYTSRLHSGVPSRFSGSGSGTDYTLTISSLQPEDFATYYCQQGYTLPLTFGQGTKVEIK

SEQ ID NO: 14 - protein, 119 aa, synthetic construct
DVQLQESGPGLVKPSQSLSLTCSVTGYSITSDFYWNWIRQFPGNKLEWMGYITYDGSTNYDPSLKNRISITRDTSKNQFFLKLNSVTAEDTATYYCVYGDFNRHAMDYWGQGTSVTVSS

SEQ ID NO: 15 - protein, 119 aa, synthetic construct
QVQLQESGPGLVKPSETLSLTCTVSGYSITSDFYWNWIRQPPGKGLEWIGYITYDGSTNYNPSLKSRVTISRDTSKNQFSLKLSSVTAADTAVYYCVYGDFNRHAMDYWGQGTLVTVSS

SEQ ID NO: 16 - protein, 111 aa, synthetic construct
DIVMSQSPSSLAVSAGEKVTMSCRSSQSLFNSRTRKNYLAWYQQKPGQPPKVLIYWASTRESGVPDRFTGSGSGTDFTLTISSVQAEDLAVYYCEQSFYLFTFGTGTKLEI

SEQ ID NO: 17 - protein, 112 aa, synthetic construct
DIVMTQSPDSLAVSLGERATINCRSSQSLFNSRTRKNYLAWYQQKPGQPPKVLIYWASTRESGVPDRFSGSGSGTDFTLTISSLQAEDVAVYYCEQSFYLFTFGQGTKVEIK

SEQ ID NO: 18 - protein, 120 aa, synthetic construct
EVHLQQSGPVLVKPGPSVKISCKASGFTFTDYYMHWVKQSHGKSLEWIGLVYPYNGDISYNQKFKGKATLTVDTSSSTAYMELNSLTSEDSAVYYCARQGNYVNNAIDYWGQGTSVTVSS

SEQ ID NO: 19 - protein, 120 aa, synthetic construct
EVQLVQSGAEVKKPGASVKVSCKASGFTFTDYYMHWVRQAPGQSLEWMGLVYPYNGDISYAQKFQGRVTLTVDTSISTAYMELSRLRSDDTAVYYCARQGNYVNNAIDYWGQGTLVTVSS

SEQ ID NO: 20 - protein, 120 aa, synthetic construct
EVQLVQSGAEVKKPGASVKVSCKASGFTFTDYYMHWVRQAPGQSLEWMGLVYPYSGDISYAQKFQGRVTLTVDTSISTAYMELSRLRSDDTAVYYCARQGNYVNNAIDYWGQGTLVTVSS

SEQ ID NO: 21 - protein, 106 aa, synthetic construct
DIVMTQSQKFMSTSVGDRVSISCKASQNVGNIIAWYQQKPGQSPKALIYLASYRYSGVPDRFTGSGSGTDFTLTINNVQSEDLAEYFCQQYSDSPYTFGSGTKLEI

SEQ ID NO: 22 - protein, 107 aa, synthetic construct
DIQMTQSPSSLSASVGDRVTITCKASQNVGNIIAWYQQKPGKSPKALIYLASYRYSGVPSRFSGSGSGTDFTLTISSLQPEDVATYFCQQYSDSPYTFGQGTKVEIK

SEQ ID NO: 23 - protein, 5 aa, synthetic construct
SHWVN

SEQ ID NO: 24 - protein, 17 aa, synthetic construct
QIYPGNGDTNYAQKFQG

SEQ ID NO: 25 - protein, 4 aa, synthetic construct
WFAY

SEQ ID NO: 26 - protein, 17 aa, synthetic construct
KSSQSLLDGGNQKNYLA

SEQ ID NO: 27 - protein, 7 aa, synthetic construct
FASIRES

SEQ ID NO: 28 - protein, 9 aa, synthetic construct
QQHYNTPWT

SEQ ID NO: 29 - protein, 8 aa, synthetic construct
GYAFSSHW

SEQ ID NO: 30 - protein, 8 aa, synthetic construct
IYPGNGDT

SEQ ID NO: 31 - protein, 6 aa, synthetic construct
ARWFAY

SEQ ID NO: 32 - protein, 12 aa, synthetic construct
QSLLDGGNQKNY

SEQ ID NO: 33 - protein, 449 aa, synthetic construct
EVQLVQSGAEVKKPGASVKVSCKASGYTFTDYYMNWVRQAPGQRLEWMGVINPYNGGTNYSQKFQGRVTLTVDKSASTAYMELSSLRSEDTAVYYCARDSNYVGLLDYWGQGTLVTVSSASTKGPSVFPLAPSSKSTSGGTAALGCLVKDYFPEPVTVSWNSGALTSGVHTFPAVLQSSGLYSLSSVVTVPSSSLGTQTYICNVNHKPSNTKVDKKVEPKSCDKTHTCPPCPAPELLGGPSVFLFPPKPKDTLMISRTPEVTCVVVDVSHEDPEVKFNWYVDGVEVHNAKTKPREEQYNSTYRVVSVLTVLHQDWLNGKEYKCKVSNKALPAPIEKTISKAKGQPREPQVYTLPPSRDELTKNQVSLTCLVKGFYPSDIAVEWESNGQPENNYKTTPPVLDSDGSFFLYSKLTVDKSRWQQGNVFSCSVMHEALHNHYTQKSLSLSPGK

SEQ ID NO: 34 - protein, 5 aa, synthetic construct
DYYMN

SEQ ID NO: 35 - protein, 17 aa, synthetic construct
VINPYNGGTNYSQKFQG

SEQ ID NO: 36 - protein, 17 aa, synthetic construct
VINPYNGGTNYAQKFQG

SEQ ID NO: 37 - protein, 10 aa, synthetic construct
DSNYVGLLDY

SEQ ID NO: 38 - protein, 11 aa, synthetic construct
RASQSISNNLH

SEQ ID NO: 39 - protein, 7 aa, synthetic construct
YASQSIS

SEQ ID NO: 40 - protein, 9 aa, synthetic construct
QQSNSWPYT

SEQ ID NO: 41 - protein, 8 aa, synthetic construct
GYTFTDYY

SEQ ID NO: 42 - protein, 8 aa, synthetic construct
INPYNGGT

SEQ ID NO: 43 - protein, 12 aa, synthetic construct
ARDSNYVGLLDY

SEQ ID NO: 44 - protein, 6 aa, synthetic construct
QSISNN

SEQ ID NO: 45 - protein, 449 aa, synthetic construct
EVQLVQSGAEVKKPGASVKVSCKASGYTFTDYYMNWVRQAPGQRLEWMGVINPYNGGTNYAQKFQGRVTLTVDKSASTAYMELSSLRSEDTAVYYCARDSNYVGLLDYWGQGTLVTVSSASTKGPSVFPLAPSSKSTSGGTAALGCLVKDYFPEPVTVSWNSGALTSGVHTFPAVLQSSGLYSLSSVVTVPSSSLGTQTYICNVNHKPSNTKVDKKVEPKSCDKTHTCPPCPAPELLGGPSVFLFPPKPKDTLMISRTPEVTCVVVDVSHEDPEVKFNWYVDGVEVHNAKTKPREEQYNSTYRVVSVLTVLHQDWLNGKEYKCKVSNKALPAPIEKTISKAKGQPREPQVYTLPPSRDELTKNQVSLTCLVKGFYPSDIAVEWESNGQPENNYKTTPPVLDSDGSFFLYSKLTVDKSRWQQGNVFSCSVMHEALHNHYTQKSLSLSPGK

SEQ ID NO: 46 - protein, 5 aa, synthetic construct
DAWMD

SEQ ID NO: 47 - protein, 19 aa, synthetic construct
EIRNKANNHATYYVDSVKG

SEQ ID NO: 48 - protein, 14 aa, synthetic construct
NNYGSTWTYYAMDY

SEQ ID NO: 49 - protein, 11 aa, synthetic construct
RASQDISNYLN

SEQ ID NO: 50 - protein, 7 aa, synthetic construct
YTSRLHS

SEQ ID NO: 51 - protein, 9 aa, synthetic construct
QQGYTLPLT

SEQ ID NO: 52 - protein, 8 aa, synthetic construct
GFTFSDAW

SEQ ID NO: 53 - protein, 10 aa, synthetic construct
IRNKANNHAT

SEQ ID NO: 54 - protein, 16 aa, synthetic construct
TRNNYGSTWTYYAMDY

SEQ ID NO: 55 - protein, 6 aa, synthetic construct
QDISNY

SEQ ID NO: 56 - protein, 214 aa, synthetic construct
DIVLTQSPATLSLSPGERATLSCRASQSISNNLHWYQQKPGQAPRLLIKYASQSISGIPARFSGSGSGPDFTLTISSLEPEDFAVYFCQQSNSWPYTFGQGTKVEIKRTVAAPSVFIFPPSDEQLKSGTASVVCLLNNFYPREAKVQWKVDNALQSGNSQESVTEQDSKDSTYSLSSTLTLSKADYEKHKVYACEVTHQGLSSPVTKSFNRGEC

SEQ ID NO: 57 - protein, 6 aa, synthetic construct
SDFYWN

SEQ ID NO: 58 - protein, 16 aa, synthetic construct
YITYDGSTNYNPSLKS

SEQ ID NO: 59 - protein, 10 aa, synthetic construct
GDFNRHAMDY

SEQ ID NO: 60 - protein, 17 aa, synthetic construct
RSSQSLFNSRTRKNYLA

SEQ ID NO: 61 - protein, 7 aa, synthetic construct
WASTRES

SEQ ID NO: 62 - protein, 8 aa, synthetic construct
EQSFYLFT

SEQ ID NO: 63 - protein, 9 aa, synthetic construct
GYSITSDFY

SEQ ID NO: 64 - protein, 7 aa, synthetic construct
ITYDGST

SEQ ID NO: 65 - protein, 12 aa, synthetic construct
VYGDFNRHAMDY

SEQ ID NO: 66 - protein, 12 aa, synthetic construct
QSLFNSRTRKNY

SEQ ID NO: 67 - protein, 450 aa, synthetic construct
EVQLVQSGAEVKKPGASVKVSCKASGFTFTDYYMHWVRQAPGQSLEWMGLVYPYNGDISYAQKFQGRVTLTVDTSISTAYMELSRLRSDDTAVYYCARQGNYVNNAIDYWGQGTLVTVSSASTKGPSVFPLAPSSKSTSGGTAALGCLVKDYFPEPVTVSWNSGALTSGVHTFPAVLQSSGLYSLSSVVTVPSSSLGTQTYICNVNHKPSNTKVDKKVEPKSCDKTHTCPPCPAPELLGGPSVFLFPPKPKDTLMISRTPEVTCVVVDVSHEDPEVKFNWYVDGVEVHNAKTKPREEQYNSTYRVVSVLTVLHQDWLNGKEYKCKVSNKALPAPIEKTISKAKGQPREPQVYTLPPSRDELTKNQVSLTCLVKGFYPSDIAVEWESNGQPENNYKTTPPVLDSDGSFFLYSKLTVDKSRWQQGNVFSCSVMHEALHNHYTQKSLSLSPGK

SEQ ID NO: 68 - protein, 5 aa, synthetic construct
DYYMH

SEQ ID NO: 69 - protein, 17 aa, synthetic construct
LVYPYNGDISYAQKFQG

SEQ ID NO: 70 - protein, 17 aa, synthetic construct
LVYPYSGDISYAQKFQG

SEQ ID NO: 71 - protein, 11 aa, synthetic construct
QGNYVNNAIDY

SEQ ID NO: 72 - protein, 11 aa, synthetic construct
KASQNVGNIIA

SEQ ID NO: 73 - protein, 7 aa, synthetic construct
LASYRYS

SEQ ID NO: 74 - protein, 9 aa, synthetic construct
QQYSDSPYT

SEQ ID NO: 75 - protein, 8 aa, synthetic construct
GFTFTDYY

SEQ ID NO: 76 - protein, 8 aa, synthetic construct
VYPYNGDI

SEQ ID NO: 77 - protein, 8 aa, synthetic construct
VYPYSGDI

SEQ ID NO: 78 - protein, 13 aa, synthetic construct
ARQGNYVNNAIDY

SEQ ID NO: 79 - protein, 6 aa, synthetic construct
QNVGNI

SEQ ID NO: 80 - protein, 450 aa, synthetic construct
EVQLVQSGAEVKKPGASVKVSCKASGFTFTDYYMHWVRQAPGQSLEWMGLVYPYSGDISYAQKFQGRVTLTVDTSISTAYMELSRLRSDDTAVYYCARQGNYVNNAIDYWGQGTLVTVSSASTKGPSVFPLAPSSKSTSGGTAALGCLVKDYFPEPVTVSWNSGALTSGVHTFPAVLQSSGLYSLSSVVTVPSSSLGTQTYICNVNHKPSNTKVDKKVEPKSCDKTHTCPPCPAPELLGGPSVFLFPPKPKDTLMISRTPEVTCVVVDVSHEDPEVKFNWYVDGVEVHNAKTKPREEQYNSTYRVVSVLTVLHQDWLNGKEYKCKVSNKALPAPIEKTISKAKGQPREPQVYTLPPSRDELTKNQVSLTCLVKGFYPSDIAVEWESNGQPENNYKTTPPVLDSDGSFFLYSKLTVDKSRWQQGNVFSCSVMHEALHNHYTQKSLSLSPGK

SEQ ID NO: 81 - protein, 214 aa, synthetic construct
DIQMTQSPSSLSASVGDRVTITCKASQNVGNIIAWYQQKPGKSPKALIYLASYRYSGVPSRFSGSGSGTDFTLTISSLQPEDVATYFCQQYSDSPYTFGQGTKVEIKRTVAAPSVFIFPPSDEQLKSGTASVVCLLNNFYPREAKVQWKVDNALQSGNSQESVTEQDSKDSTYSLSSTLTLSKADYEKHKVYACEVTHQGLSSPVTKSFNRGEC

SEQ ID NO: 82 - protein, 330 aa, synthetic construct [sequence omitted]

SEQ ID NO: 83 - protein, 107 aa, synthetic construct [sequence omitted]

SEQ ID NO: 84 - protein, 4 aa, synthetic construct
KAAD

SEQ ID NO: 85 - protein, 4 aa, unidentified
KAAN

SEQ ID NO: 86 - protein, 4 aa, synthetic construct
GGFG

SEQ ID NO: 87 - protein, 4 aa, synthetic construct
VKGG